European Patent Specification EP 3 257 939 B1, published June 14, 2023. Title: The novel Lysine Decarboxylase and Process for producing cadeverine using the same. Applicant: CJ CheilJedang Corporation. The sequence listing filed with the application follows.

SEQUENCE LISTING (24 sequences)

SEQ ID NO: 1 - protein, 751 aa, Pseudomonas thermotolerans
  PEPTIDE (1)..(751): Lysine decarboxylase from Pseudomonas thermotolerans (PtLDC)
MYKDLQFPILIVHRDIKADTVAGNRVREIARELEQDGFAILSTASASEGRIVASTHHGLACILVAAEGAGENRSLLQDVVELIRVARVRAPQLPIFALGEQVTIENAPAEAMADLNQLRGLLYLFEDTVPFLARQVARAARGYLEGLLPPFFRALVEHTAQSNYSWHTPGHGGGVAYRKSPVGQAFHQFFGENTLRSDLSVSVPELGSLLDHTGPLAEAETRAARNFGADHTYFVINGTSTANKIVWHSMVGRDDLVLVDRNCHKSILHAIIMTGAIPLYLCPERNELGIIGPIPLSEFSKEAIQAKIAASPLARGREPRVKLAVVTNSTYDGLCYNAEMVKQALGDSVEVLHFDEAWYAYAAFHEFYAGRYGMGTRLEADSPLVFATHSTHKLLAAFSQASMIHVRDGGSRKLDRYRFNEAFMMHISTSPQYSILASLDVASAMMEGPAGRSLIQETFDEALSFRRALANLRQNLPADDWWFDIWQPPRAAGVEEVATRDWLLEPNAEWHGFGEVNDDYVLLDPVKVTLVTPGLSAGGRLDEHGIPAAVVSKFLWERGLVVEKTGLYSFLVLFSMGITKGKWSTLLTELLEFKRLYDANVALAEALPSIARAGGTRYAGMGLRDLCDELHACYRENATAKALKRMYTTLPEVVMKPADAYDRLVRGEVEAVPIDRLEGRIAAVMLVPYPPGIPLIMPGERFTQATRSIIDYLGFARDFDRRFPGFDADVHGLQSEERGGERCYTVDCIKI

SEQ ID NO: 2 - DNA, 2256 bp, Pseudomonas thermotolerans
  gene (1)..(2256): Lysine decarboxylase gene from Pseudomonas thermotolerans (ptldc)
atgtacaaagacctccaattccccattctcatcgtccatcgcgacatcaaggccgataccgtggccggcaaccgcgtccgtgagatcgcccgcgaactggaacaggacggcttcgccatcctctccacggcaagtgccagcgaagggcgcatcgtcgcttccacccaccatggtctggcctgcatcctggtcgccgccgagggagcgggagagaatcgaagcctgctgcaggacgtggtggagctgatccgcgtggccagggtccgtgcgccgcagctgccgatcttcgctctcggcgagcaggtgaccatcgagaacgctccggccgaggccatggccgacctcaaccaactgcgcgggctgctctacctgttcgaggacaccgtgcccttcctcgcccgtcaggtggcgcgggccgcgcgtggctacctggaggggctgctgccgccgttcttccgcgccctggtggagcacaccgcgcagtccaactattcctggcacaccccggggcacggcggcggtgtggcttaccgcaagagcccggtggggcaggcctttcaccagttcttcggcgagaacaccctgcgctccgacttgtcggtttccgtaccggagctgggttcgctgctggatcacaccgggccgctggccgaggcggaaacccgcgcggcgcgcaacttcggcgccgaccatacctatttcgtgatcaacggcacctcgacggccaacaagatcgtctggcactccatggtcggccgcgacgatctggtgttggtggaccgcaactgccacaagtcgatcctccacgccatcatcatgaccggtgccatccccctgtacctgtgcccggagcgcaacgagctgggcatcatcgggccgattccgctctccgagttcagcaaggaggcgatccaggcgaagatcgccgccagcccgctggccagagggcgcgagccgcgggtcaagctggcggtggtgaccaattccacctacgacggcctctgttacaacgccgagatggtcaagcaggccctcggcgacagcgtcgaggtgctgcacttcgacgaggcctggtacgcctacgcggccttccacgagttctacgcggggcgttacggcatgggcactcgcctggaggcggactcgcctctggtctttgccacccattccacccacaagctgctggctgccttcagccaggcctcgatgattcacgtgcgcgacggcggtagccgcaagctggaccggtaccgcttcaacgaggccttcatgatgcacatctccacctcgccgcagtacagcatcctcgcctcgctggacgtggcctcggcgatgatggagggaccggccgggcgctcgctgatccaggaaaccttcgatgaagcgctgagcttccgccgtgctctggccaacctgcgccagaacctgccggcggacgactggtggttcgacatctggcagccgccgcgcgctgctggtgtcgaggaggtggcgacccgcgactggctgctggagccgaatgccgagtggcacggcttcggcgaggtgaacgacgactacgtgctgctcgatccggtcaaggtcaccctggtcaccccggggctgagcgccggcgggcgcctggacgagcacggcattcccgccgcggtggtcagcaagttcctctgggaacgcggcctggtggtggagaagaccggcctgtactccttcctggtgttgttctccatggggatcaccaagggcaagtggagcaccctgctcaccgagctgctggagttcaagcgcctctacgacgccaacgtggcgcttgccgaggcgttgccgagcatcgcccgcgccggtggcacccgctatgccggcatgggcctgcgcgacctgtgcgacgagctgcacgcctgctaccgggagaacgccaccgccaaggccctcaagcgcatgtacaccacgctccccgaggtggtgatgaagcctgccgatgcctacgaccggctggtccgcggagaggtggaggcggtgcccatcgaccgtctggaaggacgaatcgccgcggtgatgctggtgccctatccgccgggcattccgctgatcatgccgggcgagcgcttcacccaggcgacccgttcgatcatcgactacctgggtttcgcccgcgatttcgatcgccgcttccccggcttcgacgcggacgtgcacggcctgcagagcgaggagcgcggcggcgagcgatgctacacggtggactgcatcaagatctga

SEQ ID NO: 3 - protein, 751 aa, Pseudomonas alcaligenes
  PEPTIDE (1)..(751): Lysine decarboxylase from Pseudomonas alcaligenes (PaLDC)
MYKDLKFPILIVHRDIKADTVAGDRVRGIARELEQDGFVILSTASSAEGRIVASTHHGLACILVAAEGAGENQRLLQDVVELIRVARVRAPQLPIFALGEQVTIENAPAEAMADLNQLRGLLYLFEDTVPFLARQVARAARNYLEGLLPPFFRALVEHTAQSNYSWHTPGHGGGVAYRKSPVGQAFHQFFGENTLRSDLSVSVPELGSLLDHTGPLAEAEARAARNFGADHTFFVINGTSTANKIVWHSMVARDDLVLVDRNCHKSILHSIIMTGAIPLYLSPERNELGIIGPIPLSEFSRESIQAKIDASPLARGRAPKVKLAVVTNSTYDGLCYNAELIKQALGDTVEVLHFDEAWYAYAAFHEFYDGRYGMGTARSEEGPLVFTTHSTHKLLAAFSQASMIHVQDGGARQLDRDRFNEAFMMHISTSPQYGIIASLDVASAMMEGPAGRSLIQETFDEALSFRRALANVWQTLDAKDWWFDIWEPPQVEGAEAVATGDWVLEPGADWHGFGEVADDYVLLDPIKVTLVTPGLSADGKLGEQGIPAAVVGKFLWERGLVVEKTGLYSFLVLFSMGITKGKWSTLLTELLEFKRSYDANAPLTSALPSVARADAARYQGLGLRDLCDQLHACYRDNATAKAMRRMYTALPELAIKPSEAYDKLVRGEVEAVPIEQLQGRIAAVMLVPYPPGIPLIMPGERFTAQTRSIIDYLAFARTFDSAFPGFDSDVHGLQHDDSPMGRCYTVDCIRE

SEQ ID NO: 4 - DNA, 2256 bp, Pseudomonas alcaligenes
  gene (1)..(2256): Lysine decarboxylase gene from Pseudomonas alcaligenes (paldc)
atgtacaaagacctgaagttccccatcctcatcgtccaccgcgacatcaaggccgatacggtcgccggtgatcgcgtgcgcggcatcgcccgcgaactggagcaggacggtttcgtcatcctctccaccgccagttccgccgaagggcgcatcgtcgcctccacccaccacggcttggcctgcatcctcgtcgccgccgaaggggcgggcgagaaccagcgcctgctgcaggacgtggtcgagctgatccgcgtggcccgggtgcgtgcgccgcaactgccgatcttcgccctgggcgaacaggtgaccatcgagaacgccccggccgaagccatggccgacctcaaccagctgcgcggcctgctctacctcttcgaagacaccgtgcccttcctcgcccgccaggtcgcccgcgccgcgcgcaactacctcgaaggcctgctgccgccgttcttccgtgccctggtggagcacaccgcgcaatccaactactcctggcacacgcccggtcacggcggtggcgtcgcctaccgcaagagcccggtggggcaggccttccaccagttcttcggcgaaaacaccctgcgctcggacctctccgtctcggtgcccgagctgggctcgctgctggatcacaccggccccctggccgaagccgaggcccgcgccgcgcgcaacttcggtgctgaccacaccttcttcgtgatcaacggcacctccaccgcgaacaagatcgtctggcactccatggtcgcccgcgacgacctggtgctggtggaccgcaactgccacaagtcgatcctccactcgatcatcatgaccggcgccatcccgctctacctgagccccgagcgcaacgaactgggcatcatcgggcccatccccctgagcgagttcagtcgcgaatcgatccaggccaagatcgacgccagcccactggcccggggccgcgcgcccaaggtcaagctggcggtggtgaccaactccacctacgacggcctctgctacaacgccgagctgatcaagcaggcgctgggcgacaccgttgaggtgctgcacttcgacgaagcctggtacgcctacgccgccttccacgagttctacgacggccgctacggcatgggtacggcgcgcagcgaagaaggcccgctggtgttcaccacccactccacccacaagctgctggcggccttcagtcaggcctcgatgatccatgtgcaggacggcggcgcccgccagctggaccgggatcgcttcaacgaggcgttcatgatgcacatctccacttcgccccagtacggcatcatcgcctcgctggacgtcgcctcggcgatgatggaaggccccgccgggcgctcgctgatccaggaaaccttcgacgaggccctgagcttccgccgtgccctggccaacgtctggcagaccctggatgccaaggattggtggttcgatatctgggagccgccccaggtggaaggcgccgaggcggtggccaccggcgactgggtgctggagcccggcgccgactggcacggcttcggcgaggtggcggacgactacgtgctgctcgacccgatcaaggtcaccctggtcacccccgggctcagtgccgacggcaagctcggcgagcagggcatcccggcggcggtggtgggcaagttcctctgggagcgtggcctggtggtggagaagaccggtctctactccttcctcgtgctgttctccatgggcatcaccaagggcaaatggagcaccctgctcaccgagctgctggagttcaaacgctcctacgacgccaacgccccgctgaccagtgcactgccctcggtggcccgggccgatgccgcccgctaccaggggctgggcctgcgcgacctctgcgaccagctgcacgcctgctaccgcgacaacgccacggccaaggccatgcggcgcatgtacaccgcgcttccggagctggccatcaagccgtcggaggcttacgacaagctggtgcgtggcgaggtcgaggcggtgcccatcgagcagctgcaagggcgcattgccgcggtgatgctggtgccgtacccgccgggcatcccgctgatcatgccgggggagcgtttcactgcgcagacccgctcgatcattgactacctggccttcgcccggaccttcgacagcgccttccccggcttcgattccgatgtccacggcctgcagcacgacgacagcccaatggggcgctgctataccgttgattgcataagggagtga

SEQ ID NO: 5 - protein, 751 aa, Pseudomonas resinovorans
  PEPTIDE (1)..(751): Lysine decarboxylase from Pseudomonas resinovorans (PrLDC)
MYKELKFPVLIVHRDIKADTVAGERVRSIARELEQDGFTILPTASSAEGRIVASTHHGLACILVAAEGAGENQRLLQDMVELIRVARVRAPQLPIFALGEQVTIENAPAEAMADLNQLRGLLYLYEDTVPFLARQVARAARGYLEALLPPFFRALVEHTAQSNYSWHTPGHGGGVAYRKSPVGQAFHQFFGENTLRSDLSVSVPELGSLLDHTGPLAEAEARAAQNFGADHTFFVINGTSTANKIVWHSMVGRDDLVLVDRNCHKSIVHSIIMTGAIPLYLTPERNELGIIGPIPLAEFSRESIQAKIDASPLAKGRAAKVKLAVVTNSTYDGLCYNAELIKQALGDSVEVLHFDEAWYAYAAFHEFYAGRYGMCTHREAHSPLVFTTHSTHKLLAAFSQASMIHVQDGGARQLDRHRFNEAFMMHISTSPQYGIIASLDVASAMMEGPAGRSLIQETFDEALRFRRALANLRQNLAADDWWFDIWQSHLAEGADTVATEDWLLRPDADWHGFGDVAEDYVLLDPIKVTLVTPGLTADGKLGERGIPAAVVSKFLWERGVVVEKTGLYSFLVLFSMGITKGKWSTLLTELLEFKRGYDTNLPLAEALPSIARDHGARYAGMGLRDLCDALHGCYRNSATPKALRRMYTQLPELAMKPADAYDKLVRGEVEPVSLDLLQGRIAAVMLVPYPPGIPLIMPGERFTAETRAIIDYLEFARTFDLSFPGFDIDVHGLNCQESPTGRCYTVDCIRE

SEQ ID NO: 6 - DNA, 2256 bp, Pseudomonas resinovorans
  gene (1)..(2256): Lysine decarboxylase gene from Pseudomonas resinovorans (prldc)
atgtacaaagagctcaagttccccgtcctcatcgtccatcgtgacatcaaggccgataccgtcgccggcgagcgggtccgcagcatcgcccgcgagctggagcaggacggcttcaccatcctccccaccgccagctccgccgaaggccgtatcgtcgcctccacccaccatggcctcgcctgcatcctggtggccgccgaaggcgccggggaaaaccagcggctgctgcaggacatggtggagctgatccgcgtggcgcgggtgcgcgcgccgcagttgccgatcttcgccctgggggaacaggtcaccatcgagaacgcgccggccgaggccatggccgacctcaaccagttgcgcggcctgctctatctctacgaagacaccgtgcctttcctcgcccgccaggtggcccgagccgcccgcggctacctggaagccctgttgccgccattcttccgcgccctggtcgagcacaccgcgcagtccaactactcctggcacaccccgggccacggcggtggcgtggcctaccgcaagagtccggtggggcaggccttccaccagttcttcggggaaaacaccctgcgctcggacctctcggtatcggtgccggaactgggctcgctgctggaccacaccgggcccctggccgaagccgaggcgcgtgcggcgcagaacttcggcgccgaccacaccttcttcgtgatcaatggcacttccaccgccaacaagatcgtctggcactccatggtcggccgcgatgacctggtgctggtggaccgcaactgccacaagtccatcgtccactcgatcatcatgaccggcgccatccccctgtacctgacgccggagcgcaacgaactgggcatcatcggacccatccccctcgccgaattcagccgtgagtcgatccaggcgaagatcgacgccagccccctggccaaggggcgagccgccaaggtcaagctggcggtggtgaccaactccacctacgacggcctctgctacaacgccgagctgatcaagcaggcactgggcgactcggtggaggtgctgcacttcgacgaggcctggtacgcctacgctgccttccacgagttctatgccgggcgctacggcatgtgcacccaccgcgaggcgcactcgccgctggtcttcaccacccattccacccacaagctgctggccgccttcagccaggcctcgatgatccatgtgcaggacggcggcgcgcgccagctcgaccggcaccgcttcaacgaagccttcatgatgcacatctccacctcgccgcagtacggcatcatcgcttccctggacgtggcctcggccatgatggaggggcccgccgggcgctcgttgatccaggagactttcgacgaggcgctgcgttttcgccgcgccctggccaacctgcggcagaacctggcggcggacgactggtggttcgatatctggcagtcgcacctggcggaaggcgccgacacggtcgccaccgaggattggctgttgcgtcccgacgccgactggcacggattcggcgatgtggccgaggactacgtgctgctcgatccgatcaaggtcaccctggtgacgccgggcctgaccgccgatggcaagctgggggagcggggcattcccgcggcggtggtcagcaagttcctctgggagcgtggggtggtggtggagaagaccggcctctattccttcctggtgctgttctccatgggtatcaccaagggcaagtggagcaccctgctcaccgagttgctggagttcaagcgcggctatgacaccaacctgcccctggccgaggcgctgccctccatcgcccgggaccacggcgcgcggtacgccggcatgggcctgcgcgatctctgcgacgccctgcatggctgctaccgcaacagcgccacgcccaaggccctgcggcgcatgtacacacagctgccggaactggcgatgaagcccgccgacgcttacgacaagctggtgcgcggcgaggtggaaccggtgtccctggacctgctgcaagggcggatcgcggcggtgatgctggtgccctatccaccgggcataccgctgatcatgccgggggagcgcttcaccgccgagactcgcgcgatcatcgattacctggaattcgcccgcaccttcgacctgagcttccccggcttcgatatcgatgtgcatggcctcaactgtcaggaaagtcctaccgggcgctgctatacagtggactgcatcagggaataa

SEQ ID NO: 7 - protein, 749 aa, Pseudomonas putida
  PEPTIDE (1)..(749): Lysine decarboxylase from Pseudomonas putida (PpLDC)
MYKDLKFPILIVHRAIKADSVAGERVRGIAEELRQDGFAILAAADHAEARLVAATHHGLACMLIAAEGVGENTHLLQNMAELIRLARLRAPDLPIFALGEQVTLENAPAEAMSELNQLRGILYLFEDTVPFLARQVARAAHTYLDGLLPPFFKALVQHTAQSNYSWHTPGHGGGVAYHKSPVGQAFHQFFGENTLRSDLSVSVPELGSLLDHTGPLAEAEARAARNFGADHTFFVINGTSTANKIVWHAMVGRDDLVLVDRNCHKSVVHAIIMTGAVPLYLCPERNELGIIGPIPLSEFSPEAIEAKIQANPLARDRGRRIKLAVVTNSTYDGLCYHAGMIKQCLGASVEVLHFDEAWFAYAAFHDFFTGRYAMGTACTAGSPLVFSTHSTHKLLAAFSQASMIHVQDGARRQLDRDRFNEAFMMHISTSPQYSILASLDVASSMMEGPAGHSLLQEMFDEALSFRRALANLREHIAADDWWFSIWQPPGTEGIQRLAAQDWLLQPGAEWHGFGEVVDDYVLLDPLKVTLVMPGLSAGGVLGEHGIPAAVVSKFLWERGLVVEKTGLYSFLVLFSMGITKGKWSTLLTELLEFKRHYDGNTALSSCLPSVVAADASRYQRMGLRDLCDQLHDCYRANATAKQLKRLFTRLPEVAVSPARAYDQMVRGDVEAVPIEALLGRVAAVMLVPYPPGIPLIMPGERFTEATRSILDYLAFARAFNQGFPGFVADVHGLQNESGRYTVDCITECE

SEQ ID NO: 8 - DNA, 2250 bp, Pseudomonas putida
  gene (1)..(2250): Lysine decarboxylase gene from Pseudomonas putida (ppldc)
atgtacaaggacctcaagttcccgatcctcatcgtccaccgggctatcaaggctgacagtgtcgccggggagcgcgtgcggggcatcgccgaggaactgcgccaggacggtttcgccattctggccgccgccgaccacgccgaagcgcgcctggttgccgccactcaccacggcctggcctgcatgctgattgccgccgaaggagttggcgaaaacacccacctgctgcagaacatggccgagctgatccgcctggcgcgcatgcgcgcgcccgacttgccgatcttcgccttgggcgagcaggtgaccctggaaaacgcccctgccgaagccatgagcgagctcaaccaactgcgtggcatcctttacctgttcgaagacaccgtgccgtttctcgcccgccaggtggcgcgtgccgcacacacctaccttgacggtctgctgccaccgttcttcaaggccctggtgcagcataccgcgcagtccaactattcctggcataccccgggccatggcggtggcgtggcctatcataaaagcccggtaggccaggccttccaccagttcttcggggaaaacaccctgcgctcggacctgtctgtttcagtgccggagctgggctcgctgctcgaccacacaggccccttggccgaagccgaggccagggcggcgcgcaacttcggtgccgaccacaccttcttcgtcatcaatggcacctccacagccaacaagattgtctggcacgccatggtcggtcgcgacgacctggtgttggtggaccgcaactgccataagtcagtggtgcacgcgatcatcatgaccggcgccattccgctgtacctgtgcccagagcgcaacgagctgggcatcatcggcccgatcccgctcagcgagttcagccccgaggcaatcgaggcgaagatccaggccaacccccttgcccatggccgtgggcaacgtatcaagctggcggtagtgaccaactccacctatgacgggctgtgctaccacgccgggatgatcaagcaggccctgggtgccagcgtggaagtactgcacttcgacgaggcctggttcgcttatgcggcgtttcacggcttcttcaccgggcgctatgccatgggcactgcctgcgcagccgacagcccgttggtgttcagcacccattccacccacaagctgctggcggcgttcagccaggcctcgatgatccatgtgcaggacggggccaggcggcagctggaccgggaccgcttcaacgaagcgttcatgatgcatatctcgacttcgccgcagtacagcatccttgcctcgctggacgtggcctcgaccatgatggaagggcaggccgggcattcgctgttgcaagaaatgttcgatgaggcgctgagttttcgtcgtgccctggccaacctgcgcgagcacattgctgcggatgactggtggttcagtatttggcagccgcccagcactgaaggcatccagcccttggccgcgcaggactggctgctgcagccgggggcgcagtggcatggctttggtgaggtggcggacggctacgtgttgctcgaccctctgaaggtgaccctggtaatgccggggctgagtgcgggcggtgtgctgggtgagcgtggcatcccggcggcggtggtcagcaagtttctctgggagcgcgggctggtggtggaaaaaaccggcttgtacagcttcctggtgctgttttccatgggcatcaccaagggcaagtggagcaccttgctcaccgaactgctggagttcaagcgccactatgacggcaatacaccgctgagcagttgcctgccgagtgtgggggttgccgatgcctcacgctaccggggcatgggcctgcgcgacctgtgtgaacagttgcatgactgctaccgtgccaatgccacggccaagcagctgaagcgggtgttcacgcgtttgccggaggtggccgtgagccccgctcgggcttatgaccagatggtacgtggcgaggtggaagcggtgccgatcgaagctttgctgggccgtgtggccgcggtgatgctggtgccgtacccgcccggtattccgttgatcatgccgggagagcggttcaccgaggcgacccgctcgatacttgactacttggccttcgcccgagccttcaaccaaggctttccggggtttgtcgcggatgttcacggcctgcagaacgaaaatggccgctacaccgtggattgcatcatggaatgcgagtga

SEQ ID NO: 9 - protein, 751 aa, Pseudomonas synxantha
  PEPTIDE (1)..(751): Lysine decarboxylase from Pseudomonas synxantha (PxLDC)
MYKDLKFPILIVHRDIKADTVAGDRVRGIARELEQEGFSIFSAVDYAEGRLVASTHHGLACMLIAAEGAGENTHLLQNMVELIRLARVRAPNLPIFALGEQVTLENAPADAMSELNQLRGILYLFEDTVPFLARQVARSARTYLDGLLPPFFKALVQHTADSNYSWHTPGHGGGVAYRKSPVGQAFHQFFGENTLRSDLSVSVPELGSLLDHTGPLAEAEARAARNFGADHTFFVINGTSTANKIVWHSMVGRDDLVLVDRNCHKSVLHSIIMTGAIPLYLCPERNELGIIGPIPLSEFSPESIRAKIDASPLAYGRPPKVKLAVVTNSTYDGLCYNAELIKQQLGNSVEVLHFDEAWYAYAAFHEFFAGRYGMGTSRTPDSPLVFTTHSTHKLLAAFSQASMIHVQDGGARQLDRDRFNEAFMMHISTSPQYSIIASLDVASAMMEGPAGRSLLQEMFDEALSFRRALANLRQHIAAEDWWFSIWQPQSVAGIDRVATADWLLHPQDDWHGFGDVAEDYVLLDPIKVTLVMPGLNAGGALSDCGIPAAVVSKFLWERGLVVEKTGLYSFLVLFSMGITKGKWSTLLTELLEFKRSYDANVSLASCLPSVYAQGPVRYQGLGLRDLCDQLHSCYRSNATAKHLKRMYTVLPQIAMKPADAYDQLVRGEVEAVSIDALPGRIAAVMLVPYPPGIPLIMPGERFTESTRSIIDYLAFARTFDSSFPGFVADVHGLQHEDDGSGRRYTVDCIKG

SEQ ID NO: 10 - DNA, 2256 bp, Pseudomonas synxantha
  gene (1)..(2256): Lysine decarboxylase gene from Pseudomonas synxantha (pxldc)
atgtacaaagacctcaagttccctattcttatcgtgcaccgtgacatcaaggccgacaccgttgccggtgaccgggttcgaggcatcgccagggagttggaacaagagggcttcagtatattttctgcggtggattacgccgaagggcggttggtggcctccacccatcatggtttggcgtgcatgttgatcgcagcagaaggcgccggggaaaatacccacctgctgcaaaacatggtcgagctgatccgcctggcgcgggtaagggcacccaacctgccgatctttgccctgggtgagcaagtcacccttgaaaacgcgccggccgatgcgatgagcgagcttaaccagctacgcggcattctttatctgttcgaagacaccgtgccgttcctggcgcgccaggtcgcccgctctgcccgcacttacctggacggcctgttaccgccgttcttcaaggccttggtgcagcacaccgccgattccaattattcctggcacacccctggccatggcggtggcgtggcgtatcgtaaaagcccggtggggcaggcgtttcaccagttcttcggggagaacaccctgcgctcggacttgtctgtttctgtccctgaactgggctcgctgctcgatcataccgggcccctggccgaagccgaggcccgcgccgcgcgcaactttggcgccgaccataccttcttcgtcatcaatggcacctccaccgccaacaagatcgtctggcattccatggtcggtcgcgacgacctggtgttggtggaccgcaactgccacaagtcagtgctgcactcgatcatcatgaccggcgcgatcccgctgtatctgtgcccggagcgcaacgaactggggatcatcggcccgatccccttgagtgaattcagccccgaatcaatccgcgccaagatcgacgccagcccgttggcatatggccggccacccaaggtgaagctggcggtggtgaccaattccacctacgacggcctgtgctacaacgccgaactgatcaagcagcaattgggtaatagcgtagaggtgctgcacttcgacgaagcctggtatgcctatgcggcatttcacgagtttttcgccgggcgctatggcatgggcacctcgcgcacaccggacagcccgctggtatttaccacccactccacccacaaactgctggccgcattcagccaggcatcgatgattcatgtgcaggatggcggcgcacggcagctggaccgtgaccgtttcaacgaagccttcatgatgcacatctcgacttcaccgcaatacagcatcatcgcttcgctggatgtcgcttcggcgatgatggaaggccccgccgggcgctcgctgttgcaggaaatgttcgacgaggccctgagtttccgccgcgcgctggccaacctgcgccagcatatcgctgccgaggattggtggttttcgatctggcagccacaatcggtggcgggtatcgaccgcgttgccacggcggactggctattgcatccccaggatgattggcacggctttggcgatgtggctgaagattatgtcttgctggacccgatcaaagtcaccctggtgatgcctggcctcaatgcaggtggcgccttgagcgattgtgggattcccgccgcggtggtcagcaagtttctctgggagcgcggcctcgtggtggaaaaaaccgggctttattcgttcctcgtgttgttttccatggggatcaccaaaggcaagtggagcaccttgctcaccgagttgctggagttcaagcgcagttacgatgccaacgtcagcctggccagttgtttgccctcggtgtacgcccaggggccggtacgttatcagggcttgggcctgcgcgatctttgcgaccagttgcacagctgttaccgtagcaacgccaccgccaagcatctcaagcgcatgtacacagtattgccgcagatcgcgatgaaacccgccgatgcctacgaccaactggtcagaggcgaagttgaagcggtatccatcgatgccttgccaggacgcatcgcagccgtaatgctggtgccttatccaccgggcattccattgataatgcccggcgagcgctttactgaatcaacgcgttcaatcatcgactacctggcatttgcccgcacgttcgatagcagtttccccggttttgtcgccgatgttcatgggctgcaacacgaagatgatggcagtggccgtcgttacaccgtcgattgcatcaagggttaa

SEQ ID NO: 11 - protein, 715 aa, Escherichia coli
  PEPTIDE (1)..(715): Lysine decarboxylase from Escherichia coli (EcLDC)
MNVIAILNHMGVYFKEEPIRELHRALERLNFQIVYPNDRDDLLKLIENNARLCGVIFDWDKYNLELCEEISKMNENLPLYAFANTYSTLDVSLNDLRLQISFFEYALGAAEDIANKIKQTTDEYINTILPPLTKALFKYVREGKYTFCTPGHMGGTAFQKSPVGSLFYDFFGPNTMKSDISISVSELGSLLDHSGPHKEAEQYIARVFNADRSYMVTNGTSTANKIVGMYSAPAGSTILIDRNCHKSLTHLMMMSDVTPIYFRPTRNAYGILGGIPQSEFQHATIAKRVKETPNATWPVHAVITNSTYDGLLYNTDFIKKTLDVKSIHFDSAWVPYTNFSPIYEGKCGMSGGRVEGKVIYETQSTHKLLAAFSQASMIHVKGDVNEETFNEAYMMHTTTSPHYGIVASTETAAAMMKGNAGKRLINGSIERAIKFRKEIKRLRTESDGWFFDVWQPDHIDTTECWPLRSDSTWHGFKNIDNEHMYLDPIKVTLLTPGMEKDGTMSDFGIPASIVAKYLDEHGIVVEKTGPYNLLFLFSIGIDKTKALSLLRALTDFKRAFDLNLRVKNMLPSLYREDPEFYENMRIQELAQNIHKLIVHHNLPDLMYRAFEVLPTMVMTPYAAFQKELHGMTEEVYLDEMVGRINANMILPYPPGVPLVMPGEMITEESRPVLEFLQMLCEIGAHYPGFETDIHGAYRQADGRYTVKVLKEESKK

SEQ ID NO: 12 - protein, 31 aa, Artificial Sequence
  15 amino acid of Lysine decarboxylase from Escherichia coli
GRVEGKVIYETQSTHKLLAAFSQASMIHVKG

SEQ ID NO: 13 - DNA, 33 bp, Artificial Sequence
  5 LDC NdeI
aatatacatatgtacaaagacctccaattcccc

SEQ ID NO: 14 - DNA, 35 bp, Artificial Sequence
  3 LDC XhoI
aatatactcgagtcagatcttgatgcagtccaccg

SEQ ID NO: 15 - DNA, 34 bp, Artificial Sequence
  5 LDC BamHI
aatataggatccgtacaaagacctccaattcccc

SEQ ID NO: 16 - DNA, 35 bp, Artificial Sequence
  3 LDC SacI
aatatagagctctcagatcttgatgcagtccaccg

SEQ ID NO: 17 - DNA, 37 bp, Artificial Sequence
  5 PaLDC NdeI
aatatacatatgtacaaagacctgaagttccccatcc

SEQ ID NO: 18 - DNA, 41 bp, Artificial Sequence
  3 PaLDC XhoI
aatatactcgagtcactcccttatgcaatcaacggtatagc

SEQ ID NO: 19 - DNA, 39 bp, Artificial Sequence
  5 PrLDC NdeI
aatatacatatgtacaaagagctcaagttccccgtcctc

SEQ ID NO: 20 - DNA, 41 bp, Artificial Sequence
  3 PrLDC XhoI
aatatactcgagttattccctgatgcagtccactgtatagc

SEQ ID NO: 21 - DNA, 33 bp, Artificial Sequence; identical to SEQ ID NO: 13
  5_LDC_NdeI_ppldc

SEQ ID NO: 22 - DNA, 41 bp, Artificial Sequence; identical to SEQ ID NO: 18
  3_PaLDC_XhoI_ppldc

SEQ ID NO: 23 - DNA, 33 bp, Artificial Sequence; identical to SEQ ID NO: 13
  5_LDC_NdeI_pxldc

SEQ ID NO: 24 - DNA, 41 bp, Artificial Sequence; identical to SEQ ID NO: 18
  3_PaLDC_XhoI_pxldc